European Patent Specification EP 3 390 454 B1, published February 4, 2026. Title: A RECOMBINANT BI-SPECIFIC POLYPEPTIDE FOR COORDINATELY ACTIVATING TUMOR-REACTIVE T CELLS AND NEUTRALIZING IMMUNE SUPPRESSION. Applicant: University of Maryland Baltimore County Ostrand-Rosenberg, Suzanne Carter, Darryl L. The sequence listing filed with the application follows.

SEQUENCE LISTING (16 sequences)

SEQ ID NO: 1 - DNA, 318 bp, Artificial Sequence
  Synthetic construct
gaaattgtgttgacacagtctccagccaccctgtctttgtctccaggggaaagagccaccctctcctgcagggccagtcagagtgttagcagctacttagcctggtaccaacagaaacctggccaggctcccaggctcctcatctatgatgcatccaacagggccactggcatcccagccaggttcagtggcagtgggtctgggacagacttcactctcaccatcagcagcctagagcctgaagattttgcagtttattactgtcagcagcgtagcaactggccgacgttcggccaagggaccaaggtggaaatcaaa

SEQ ID NO: 2 - DNA, 369 bp, Artificial Sequence
  Synthetic construct
caggtccaactggtgcagtctggggctgaggtcaagaagcctgggtcgtcggtgaaggtctcctgcaagacttctggagacaccttcagcacctatgctatcagctgggtgcgacaggcccctggacaagggcttgagtggatgggagggatcatccctatatttggtaaagcacactacgcacagaagttccagggcagagtcacgattaccgcggacgaatccacgagcacagcctacatggagctgagcagcctgagatctgaggacacggccgtgtatttttgtgcgagaaagtttcactttgtttcggggagccccttcggtatggacgtctggggccaagggaccacggtcaccgtctcctca

SEQ ID NO: 3 - DNA, 318 bp, Artificial Sequence
  Synthetic construct
gacattcagctgacccagtctccagcaatcatgtctgcatctccaggggagaaggtcaccatgacctgcagagccagttcaagtgtaagttacatgaactggtaccagcagaagtcaggcacctcccccaaaagatggatttatgacacatccaaagtggcttctggagtcccttatcgcttcagtggcagtgggtctgggacctcatactctctcacaatcagcagcatggaggctgaagatgctgccacttattactgccaacagtggagtagtaacccgctcacgttcggtgctgggaccaagctggagctgaaa

SEQ ID NO: 4 - DNA, 363 bp, Artificial Sequence
  Synthetic construct
gatatcaaactgcagcagtcaggggctgaactggcaagacctggggcctcagtgaagatgtcctgcaagacttctggctacacctttactaggtacacgatgcactgggtaaaacagaggcctggacagggtctggaatggattggatacattaatcctagccgtggttatactaattacaatcagaagttcaaggacaaggccacattgactacagacaaatcctccagcacagcctacatgcaactgagcagcctgacatctgaggactctgcagtctattactgtgcaagatattatgatgatcattactgccttgactactggggccaaggcaccactctcacagtctcctcagtcgaa

SEQ ID NO: 5 - protein, 106 aa, Artificial Sequence
  Synthetic construct
EIVLTQSPATLSLSPGERATLSCRASQSVSSYLAWYQQKPGQAPRLLIYDASNRATGIPARFSGSGSGTDFTLTISSLEPEDFAVYYCQQRSNWPTFGQGTKVEIK

SEQ ID NO: 6 - protein, 123 aa, Artificial Sequence
  Synthetic construct
QVQLVQSGAEVKKPGSSVKVSCKTSGDTFSTYAISWVRQAPGQGLEWMGGIIPIFGKAHYAQKFQGRVTITADESTSTAYMELSSLRSEDTAVYFCARKFHFVSGSPFGMDVWGQGTTVTVSS

SEQ ID NO: 7 - protein, 106 aa, Artificial Sequence
  Synthetic construct
DIQLTQSPAIMSASPGEKVTMTCRASSSVSYMNWYQQKSGTSPKRWIYDTSKVASGVPYRFSGSGSGTSYSLTISSMEAEDAATYYCQQWSSNPLTFGAGTKLELK

SEQ ID NO: 8 - protein, 121 aa, Artificial Sequence
  Synthetic construct
DIKLQQSGAELARPGASVKMSCKTSGYTFTRYTMHWVKQRPGQGLEWIGYINPSRGYTNYNQKFKDKATLTTDKSSSTAYMQLSSLTSEDSAVYYCARYYDDHYCLDYWGQGTTLTVSSVE

SEQ ID NO: 9 - DNA, 1533 bp, Artificial Sequence
  Synthetic construct
atgggatggagctgtatcatcctcttcttggtagcaacagctacaggtgtccactccgaaattgtgttgacacagtctccagccaccctgtctttgtctccaggggaaagagccaccctctcctgcagggccagtcagagtgttagcagctacttagcctggtaccaacagaaacctggccaggctcccaggctcctcatctatgatgcatccaacagggccactggcatcccagccaggttcagtggcagtgggtctgggacagacttcactctcaccatcagcagcctagagcctgaagattttgcagtttattactgtcagcagcgtagcaactggccgacgttcggccaagggaccaaggtggaaatcaaaggtggaggtggatctgggggaggtggatctgggggtgggggatcgcaggtccaactggtgcagtctggggctgaggtcaagaagcctgggtcgtcggtgaaggtctcctgcaagacttctggagacaccttcagcacctatgctatcagctgggtgcgacaggcccctggacaagggcttgagtggatgggagggatcatccctatatttggtaaagcacactacgcacagaagttccagggcagagtcacgattaccgcggacgaatccacgagcacagcctacatggagctgagcagcctgagatctgaggacacggccgtgtatttttgtgcgagaaagtttcactttgtttcggggagccccttcggtatggacgtctggggccaagggaccacggtcaccgtctcctcaggaggtggtggatccgatatcaaactgcagcagtcaggggctgaactggcaagacctggggcctcagtgaagatgtcctgcaagacttctggctacacctttactaggtacacgatgcactgggtaaaacagaggcctggacagggtctggaatggattggatacattaatcctagccgtggttatactaattacaatcagaagttcaaggacaaggccacattgactacagacaaatcctccagcacagcctacatgcaactgagcagcctgacatctgaggactctgcagtctattactgtgcaagatattatgatgatcattactgccttgactactggggccaaggcaccactctcacagtctcctcagtcgaaggtggaagtggaggttctggtggaagtggaggttcaggtggagtcgacgacattcagctgacccagtctccagcaatcatgtctgcatctccaggggagaaggtcaccatgacctgcagagccagttcaagtgtaagttacatgaactggtaccagcagaagtcaggcacctcccccaaaagatggatttatgacacatccaaagtggcttctggagtcccttatcgcttcagtggcagtgggtctgggacctcatactctctcacaatcagcagcatggaggctgaagatgctgccacttattactgccaacagtggagtagtaacccgctcacgttcggtgctgggaccaagctggagctgaaa

SEQ ID NO: 10 - protein, 492 aa, Artificial Sequence
  Synthetic construct
EIVLTQSPATLSLSPGERATLSCRASQSVSSYLAWYQQKPGQAPRLLIYDASNRATGIPARFSGSGSGTDFTLTISSLEPEDFAVYYCQQRSNWPTFGQGTKVEIKGGGGSGGGGSGGGGSQVQLVQSGAEVKKPGSSVKVSCKTSGDTFSTYAISWVRQAPGQGLEWMGGIIPIFGKAHYAQKFQGRVTITADESTSTAYMELSSLRSEDTAVYFCARKFHFVSGSPFGMDVWGQGTTVTVSSGGGGSDIKLQQSGAELARPGASVKMSCKTSGYTFTRYTMHWVKQRPGQGLEWIGYINPSRGYTNYNQKFKDKATLTTDKSSSTAYMQLSSLTSEDSAVYYCARYYDDHYCLDYWGQGTTLTVSSVEGGSGGSGGSGGSGGVDDIQLTQSPAIMSASPGEKVTMTCRASSSVSYMNWYQQKSGTSPKRWIYDTSKVASGVPYRFSGSGSGTSYSLTISSMEAEDAATYYCQQWSSNPLTFGAGTKLELK

SEQ ID NO: 11 - DNA, 45 bp, Artificial Sequence
  Synthetic construct
ggtggaggtggatctgggggaggtggatctgggggtgggggatcg

SEQ ID NO: 12 - protein, 15 aa, Artificial Sequence
  Synthetic Construct
GGGGSGGGGSGGGGS

SEQ ID NO: 13 - DNA, 15 bp, Artificial Sequence
  Synthetic construct
ggaggtggtggatcc

SEQ ID NO: 14 - protein, 5 aa, Artificial Sequence
  Synthetic construct
GGGGS

SEQ ID NO: 15 - DNA, 48 bp, Artificial Sequence
  Synthetic construct
ggtggaagtggaggttctggtggaagtggaggttcaggtggagtcgac

SEQ ID NO: 16 - protein, 16 aa, Artificial Sequence
  Synthetic construct
GGSGGSGGSGGSGGVD